European Patent Application EP 4 431 613 A1, published September 18, 2024. Title: Method for the production of D-tagatose using a novel L-arabinose isomerase from Lentilactobacillus parakefiri. Applicant: Universität Hohenheim. The sequence listing filed with the application follows.

SEQUENCE LISTING (3 sequences)

SEQ ID NO: 1 - protein, 474 aa, Lentilactobacillus parakefiri
MLQVPDYEFWFVTGSQHLYGEEQLKSVEKDARDMVDKLNASKKLPYPIVFKMVATTADSITQLMKDVNYNDKVAGVITWMHTFSPAKNWIRGTKLLQKPLLHLATQYLDHIPYDTIDFDYMNLNQSAHGDREYGFINARLQKHNKIVYGWWGDPEVQDEIADWEDVAVAYDESFKIKVARFGDNMRNVAVTEGDKVEAQIQFGWTVDYFALGDLVESVNAVSESDIDKKYKELQDKYEFVQGDNDKDKYEHSVRYQIREYFGIKNFLDKGNYSAFTTNFEDLYGLEQLPGLAAQLLMDEGYGFGAEGDWKTAALDRLVKILTHNQATAFMEDYTLELQKGKEAILGSHMLEVDPGIASDKPRVEVHPLDIGGKADPARLVFTGREGDAMDITISDFGTEYRMIGYAVEGHKAPKPTPHLPVAKQMWTPKMGLKHGATQWIHDGGGHHTVLTFAANETQIQDLATMFGLTFNDIK

SEQ ID NO: 2 - DNA, 1425 bp, Lentilactobacillus parakefiri
  source 1..1425: mol_type = genomic DNA
atgttacaagtacctgattatgaattttggtttgttactggtagtcaacatctttacggagaagaacaattaaagtccgttgaaaaagatgcccgagacatggttgataagttgaatgcttcaaagaagcttccttacccaatcgtgttcaagatggttgccaccactgctgacagcatcactcagttaatgaaagatgttaactacaatgataaagtagccggtgttattacttggatgcacacattctcaccagctaaaaactggatccgtggtactaagttattgcaaaagccattacttcacttggcaactcaatacttggatcacattccatatgacactatcgactttgactacatgaaccttaaccaaagtgctcatggtgaccgtgaatacggctttatcaatgctcgtcttcaaaaacacaacaagatcgtttacggctggtggggagatccagaagtccaagacgaaattgctgactgggaagatgtcgcagttgcttatgacgaaagcttcaagatcaaggttgctcgtttcggtgataacatgcgtaacgttgctgttactgaaggtgacaaagttgaagctcaaatccaatttggctggaccgttgattacttcgcacttggtgacttggtagaatcagttaacgctgtttctgaaagtgacattgacaagaagtacaaagaattacaagacaagtatgaatttgtacaaggcgacaatgacaaagacaagtacgaacattcagttcgttaccaaatccgtgaatacttcggaatcaagaacttcttggacaaaggtaactactcagcattcactaccaacttcgaagacctttatggtttggaacaattacctggtcttgcagctcaattgcttatggacgaaggttatggtttcggtgccgaaggtgactggaagacagccgctcttgaccgcttagttaagatcttgactcataatcaagctactgcattcatggaagactacactcttgaattacaaaagggtaaggaagctatccttggatcacacatgcttgaagttgaccctggtattgccagtgacaagcctcgtgttgaagttcacccattggacatcggtggtaaagctgatcctgcacgtctggtatttactggtcgtgaaggcgacgcaatggacatcaccatttctgacttcggtactgaataccgtatgatcggatatgctgttgaaggacacaaagctccaaagccaactccacatcttccagttgcaaaacaaatgtggactccaaagatgggcttgaagcatggtgctactcaatggattcatgatggtggtggacaccacactgtcttgacatttgctgctaacgaaactcaaatccaagacttagctactatgtttggattgacatttaacgacatcaagtaa

SEQ ID NO: 3 - DNA, 1425 bp, synthetic construct
  source 1..1425: mol_type = other DNA
atgctgcaggttccggattatgaattttggtttgttaccggtagccagcatctgtatggtgaagaacagctgaaaagcgttgaaaaagatgcacgtgatatggtggataaactgaacgcaagcaaaaaactgccgtatccgattgtgtttaaaatggttgccaccaccgcagatagcattacccagctgatgaaagatgtgaactataacgataaagtggcaggcgttattacctggatgcatacctttagtccggcaaaaaattggattcgtggcaccaaactgctgcagaaaccgctgctgcatctggcaacccagtatctggatcatattccgtatgataccatcgacttcgattacatgaatctgaatcagagcgcacatggtgatcgtgaatatggttttatcaatgcacgcctgcagaagcacaacaaaattgtttatggttggtggggtgatccggaagttcaggatgaaattgcagattgggaagatgttgcagttgcctatgatgaaagcttcaaaatcaaagttgcccgttttggtgataacatgcgtaatgttgccgttaccgaaggtgataaagttgaagcacagattcagtttggttggaccgttgattattttgcactgggtgatctggttgaaagcgttaatgcagttagcgaaagcgatatcgacaagaaatacaaagaactgcaggacaaatatgaattcgtgcagggcgataacgacaaagataaatatgaacattcagtgcgctatcagatccgcgaatattttggcattaaaaactttctggacaaaggcaactatagcgcctttaccaccaattttgaagatctgtacggtctggaacagctgcctggtctggcagcacagctgctgatggatgaaggttatggttttggtgcagaaggtgattggaaaaccgcagcactggatcgtctggttaaaattctgacccataatcaggcaaccgccttcatggaagattacaccctggaactgcagaaaggtaaagaagcaattctgggtagccacatgctggaagttgatccgggtattgcaagcgataaaccgcgtgttgaagttcatccgctggatattggtggcaaagcagatccggcacgtctggtgtttaccggtcgtgaaggtgatgcaatggatattaccattagcgattttggcaccgaatatcgcatgattggttatgcagttgaaggtcataaagcaccgaaaccgacaccgcatctgccggttgcaaaacaaatgtggaccccgaaaatgggtctgaaacatggtgcgacccagtggattcatgatggtggtggtcatcataccgttctgacctttgcagcaaatgaaacccagattcaggatctggcgaccatgtttggcctgacctttaatgatatcaaataa